European Patent Specification EP 3 459 973 B1, published August 20, 2025. Title: Anti-Human PD-L1 Humanized Monoclonal Antibody and Its Applications. Applicant: REYOUNG (SUZHOU) BIOLOGY SCIENCE & TECHNOLOGY CO., LTD. The sequence listing filed with the application follows.

SEQUENCE LISTING (56 sequences)

SEQ ID NO: 1 - DNA, 363 bp, Artificial Sequence
aaggtccagctgcagcagtctggagctgagctggtgaaacccggggcatcagtgaagctgtcctgcaaggcttctggctacaccttcactaaatatattatacactggataaagcagaggtctggacagggtcttgagtggattgggtggttttaccctggaagtggtaatatcaggtacaatgagaaaatcaagggcaaggccacattgactgcggacaaatcctccagcacagtctatatggagcttagtggattgacatctgaggactctgcggtctatttctgtgcaagacacggggaactgggaggcggttacttctttgactactggggccaaggcaccactctcacggtctcctca

SEQ ID NO: 2 - protein, 107 aa, Artificial Sequence
QIVLSQSPTILSASPGEKVTMTCRASSSVSNIHWYQQKTGSSPKPWIYATSNLASGAPVRFSGSGSGTSYSLTISRVEAEDAATYYCQQWSSNPLTFGPGTKLELKR

SEQ ID NO: 3 - DNA, 321 bp, Artificial Sequence
caaattgttctctcccagtctccaacaatcctgtctgcatctccaggggagaaggtcacaatgacttgcagggccagctccagtgtaagtaacatacactggtaccagcagaagacaggatcctcccccaaaccctggatttatgccacatccaacctggcttctggagcccctgttcgcttcagtggcagtgggtctgggacctcttattctctcacaatcagcagagtggaggctgaagatgctgccacttattactgccagcagtggagtagtaacccactcacgttcggtcctgggaccaagctggagctgaaacgg

SEQ ID NO: 4 - protein, 121 aa, Artificial Sequence
KVQLQQSGAELVKPGASVKLSCKASGYTFTKYIIHWIKQRSGQGLEWIGWFYPGSGNIRYNEKIKGKATLTADKSSSTVYMELSGLTSEDSAVYFCARHGELGGGYFFDYWGQGTTLTVSS

SEQ ID NO: 5 - DNA, 363 bp, Artificial Sequence
gaggtgcagctggtgcagagcggcgccgaggtgaagaaacctggcgcctccgtgaaggtgagctgcaaggcctccggctacaccttcaccaagtacatcatccactgggtgcggcaagcccctggacagggactggaatggatgggctggttctaccctggttctggcaacatccggtacaacgagaagatcaagggcagggtgaccatgacccgggacaccagcacctccaccgtgtacatggagctgtcctccctgaggagcgaggacaccgccgtgtattactgcgctaggcacggagagctgggcggaggctacttcttcgactactggggccagggcacaaccgtgaccgtgtcctcc

SEQ ID NO: 6 - protein, 121 aa, Artificial Sequence
EVQLVQSGAEVKKPGASVKVSCKASGYTFTKYIIHWVRQAPGQGLEWMGWFYPGSGNIRYNEKIKGRVTMTRDTSTSTVYMELSSLRSEDTAVYYCARHGELGGGYFFDYWGQGTTVTVSS

SEQ ID NO: 7 - DNA, 321 bp, Artificial Sequence
gatatccagctgacccagagcccctcctttctgtccgcctccgtgggcgacagggtgaccatcacctgcagggccagctccagcgtgagcaacatccactggtatcaacagaagcctggcaaggcccccaagccctggatctacgccacctccaacctggccagcggcgtgcctagcaggttcagcggttctggctccggcaccgagttcaccctgaccatctcctccctgcagcccgaggacttcgccacctactactgccagcagtggtccagcaaccccctgacctttggccagggcaccaagctggagatcaagagg

SEQ ID NO: 8 - protein, 107 aa, Artificial Sequence
DIQLTQSPSFLSASVGDRVTITCRASSSVSNIHWYQQKPGKAPKPWIYATSNLASGVPSRFSGSGSGTEFTLTISSLQPEDFATYYCQQWSSNPLTFGQGTKLEIKR

SEQ ID NO: 9 - DNA, 1359 bp, Artificial Sequence
gaggtgcagctggtgcagagcggcgccgaggtgaagaaacctggcgcctccgtgaaggtgagctgcaaggcctccggctacaccttcaccaagtacatcatccactgggtgcggcaagcccctggacagggactggaatggatgggctggttctaccctggttctggcaacatccggtacaacgagaagatcaagggcagggtgaccatgacccgggacaccagcacctccaccgtgtacatggagctgtcctccctgaggagcgaggacaccgccgtgtattactgcgctaggcacggagagctgggcggaggctacttcttcgactactggggccagggcacaaccgtgaccgtgtcctccgccagcaccaagggaccatccgtgttcccactggctccaagctctaaatccactagcggaggcaccgcagccctgggatgtctggtgaaggattacttcccagagcccgtcacagtgtcatggaactccggggctctgacctctggtgtccacacatttccagcagtgctgcagagttcaggcctgtactccctgtccagcgtggtcacagtgccctctagttcactgggaactcagacctatatctgcaacgtgaatcacaagccatccaatactaaagtcgacaagaaagtggagcccaagagctgtgataaaacacatacttgccccccttgtcctgcaccagaactgctgggaggaccatccgtgttcctgtttccacccaagcctaaagacactctgatgatttctcgaacacccgaggtcacttgcgtggtcgtggacgtgtcccacgaggatcctgaagtcaagtttaactggtacgtggatggagtcgaagtgcataatgctaagacaaaacctagagaggaacagtacgccagtacatatagagtcgtgtcagtcctgactgtgctgcatcaggactggctgaacgggaaggagtataagtgcaaagtgtccaataaggctctgcccgcacctatcgagaaaactattagcaaggctaaaggccagcctagggaaccacaggtgtacaccctgcctccatctcgggaggaaatgactaagaaccaggtcagtctgacctgtctggtgaaaggcttctatccttccgacatcgcagtggagtgggaaagcaatggacagccagagaacaattacaagaccacaccccctgtgctggacagcgatgggtctttctttctgtatagtaagctgaccgtggataaatcacggtggcagcagggtaatgtcttttcttgtagtgtgatgcacgaagccctgcacaaccattacactcagaaatccctgtcactgtcccctggaaagtgataa

SEQ ID NO: 10 - protein, 401 aa, Artificial Sequence
FYPGSGNIRYNEKIKGRVTMTRDTSTSTVYMELSSLRSEDTAVYYCARHGELGGGYFFDYWGQGTTVTVSSASTKGPSVFPLAPSSKSTSGGTAALGCLVKDYFPEPVTVSWNSGALTSGVHTFPAVLQSSGLYSLSSVVTVPSSSLGTQTYICNVNHKPSNTKVDKKVEPKSCDKTHTCPPCPAPELLGGPSVFLFPPKPKDTLMISRTPEVTCVVVDVSHEDPEVKFNWYVDGVEVHNAKTKPREEQYASTYRVVSVLTVLHQDWLNGKEYKCKVSNKALPAPIEKTISKAKGQPREPQVYTLPPSREEMTKNQVSLTCLVKGFYPSDIAVEWESNGQPENNYKTTPPVLDSDGSFFLYSKLTVDKSRWQQGNVFSCSVMHEALHNHYTQKSLSLSPGK

SEQ ID NO: 11 - DNA, 15 bp, Artificial Sequence
aagtacatcatccac

SEQ ID NO: 12 - DNA, 51 bp, Artificial Sequence
tggttctaccctggttctggcaacatccggtacaacgagaagatcaagggc

SEQ ID NO: 13 - DNA, 36 bp, Artificial Sequence
cacggagagctgggcggaggctacttcttcgactac

SEQ ID NO: 14 - DNA, 90 bp, Artificial Sequence
gaggtgcagctggtgcagagcggcgccgaggtgaagaaacctggcgcctccgtgaaggtgagctgcaaggcctccggctacaccttcacc

SEQ ID NO: 15 - DNA, 42 bp, Artificial Sequence
tgggtgcggcaagcccctggacagggactggaatggatgggc

SEQ ID NO: 16 - DNA, 96 bp, Artificial Sequence
agggtgaccatgacccgggacaccagcacctccaccgtgtacatggagctgtcctccctgaggagcgaggacaccgccgtgtattactgcgctagg

SEQ ID NO: 17 - DNA, 33 bp, Artificial Sequence
tggggccagggcacaaccgtgaccgtgtcctcc

SEQ ID NO: 18 - protein, 5 aa, Artificial Sequence
KYIIH

SEQ ID NO: 19 - protein, 17 aa, Artificial Sequence
WFYPGSGNIRYNEKIKG

SEQ ID NO: 20 - protein, 12 aa, Artificial Sequence
HGELGGGYFFDY

SEQ ID NO: 21 - protein, 30 aa, Artificial Sequence
EVQLVQSGAEVKKPGASVKVSCKASGYTFT

SEQ ID NO: 22 - protein, 14 aa, Artificial Sequence
WVRQAPGQGLEWMG

SEQ ID NO: 23 - protein, 32 aa, Artificial Sequence
RVTMTRDTSTSTVYMELSSLRSEDTAVYYCAR

SEQ ID NO: 24 - protein, 11 aa, Artificial Sequence
WGQGTTVTVSS

SEQ ID NO: 25 - DNA, 642 bp, Artificial Sequence
gatatccagctgacccagagcccctcctttctgtccgcctccgtgggcgacagggtgaccatcacctgcagggccagctccagcgtgagcaacatccactggtatcaacagaagcctggcaaggcccccaagccctggatctacgccacctccaacctggccagcggcgtgcctagcaggttcagcggttctggctccggcaccgagttcaccctgaccatctcctccctgcagcccgaggacttcgccacctactactgccagcagtggtccagcaaccccctgacctttggccagggcaccaagctggagatcaagaggactgtggctgcaccatctgtcttcatcttcccgccatctgatgagcagttgaaatctggaactgcctctgttgtgtgcctgctgaataacttctatcccagagaggccaaagtacagtggaaggtggataacgccctccaatcgggtaactcccaggagagtgtcacagagcaggacagcaaggacagcacctacagcctcagcagcaccctgacgctgagcaaagcagactacgagaaacacaaagtctacgcctgcgaagtcacccatcagggcctgagctcgcccgtcacaaagagcttcaacaggggagagtgttaa

SEQ ID NO: 26 - protein, 213 aa, Artificial Sequence
DIQLTQSPSFLSASVGDRVTITCRASSSVSNIHWYQQKPGKAPKPWIYATSNLASGVPSRFSGSGSGTEFTLTISSLQPEDFATYYCQQWSSNPLTFGQGTKLEIKRTVAAPSVFIFPPSDEQLKSGTASVVCLLNNFYPREAKVQWKVDNALQSGNSQESVTEQDSKDSTYSLSSTLTLSKADYEKHKVYACEVTHQGLSSPVTKSFNRGEC

SEQ ID NO: 27 - DNA, 30 bp, Artificial Sequence
agggccagctccagcgtgagcaacatccac

SEQ ID NO: 28 - DNA, 21 bp, Artificial Sequence
gccacctccaacctggccagc

SEQ ID NO: 29 - DNA, 27 bp, Artificial Sequence
cagcagtggtccagcaaccccctgacc

SEQ ID NO: 30 - DNA, 69 bp, Artificial Sequence
gatatccagctgacccagagcccctcctttctgtccgcctccgtgggcgacagggtgaccatcacctgc

SEQ ID NO: 31 - DNA, 45 bp, Artificial Sequence
tggtatcaacagaagcctggcaaggcccccaagccctggatctac

SEQ ID NO: 32 - DNA, 96 bp, Artificial Sequence
ggcgtgcctagcaggttcagcggttctggctccggcaccgagttcaccctgaccatctcctccctgcagcccgaggacttcgccacctactactgc

SEQ ID NO: 33 - DNA, 33 bp, Artificial Sequence
tttggccagggcaccaagctggagatcaagagg

SEQ ID NO: 34 - protein, 10 aa, Artificial Sequence
RASSSVSNIH

SEQ ID NO: 35 - protein, 7 aa, Artificial Sequence
ATSNLAS

SEQ ID NO: 36 - protein, 9 aa, Artificial Sequence
QQWSSNPLT

SEQ ID NO: 37 - protein, 23 aa, Artificial Sequence
DIQLTQSPSFLSASVGDRVTITC

SEQ ID NO: 38 - protein, 15 aa, Artificial Sequence
WYQQKPGKAPKPWIY

SEQ ID NO: 39 - protein, 32 aa, Artificial Sequence
GVPSRFSGSGSGTEFTLTISSLQPEDFATYYC

SEQ ID NO: 40 - protein, 11 aa, Artificial Sequence
FGQGTKLEIKR

SEQ ID NO: 41 - DNA, 642 bp, Artificial Sequence
gatatccagctgacccagagcccctcctttctgtccgcctccgtgggcgacagggtgaccatcacctgcagggccagctccaagacggggaacatccactggtatcaacagaagcctggcaaggcccccaagccctggatctacgccacctccaacctggccagcggcgtgcctagcaggttcagcggttctggctccggcaccgagttcaccctgaccatctcctccctgcagcccgaggacttcgccacctactactgccagcagtggtccagcaaccccctgacctttggccagggcaccaagctggagatcaagaggactgtggctgcaccatctgtcttcatcttcccgccatctgatgagcagttgaaatctggaactgcctctgttgtgtgcctgctgaataacttctatcccagagaggccaaagtacagtggaaggtggataacgccctccaatcgggtaactcccaggagagtgtcacagagcaggacagcaaggacagcacctacagcctcagcagcaccctgacgctgagcaaagcagactacgagaaacacaaagtctacgcctgcgaagtcacccatcagggcctgagctcgcccgtcacaaagagcttcaacaggggagagtgttaa

SEQ ID NO: 42 - protein, 213 aa, Artificial Sequence
DIQLTQSPSFLSASVGDRVTITCRASSKTGNIHWYQQKPGKAPKPWIYATSNLASGVPSRFSGSGSGTEFTLTISSLQPEDFATYYCQQWSSNPLTFGQGTKLEIKRTVAAPSVFIFPPSDEQLKSGTASVVCLLNNFYPREAKVQWKVDNALQSGNSQESVTEQDSKDSTYSLSSTLTLSKADYEKHKVYACEVTHQGLSSPVTKSFNRGEC

SEQ ID NO: 43 - DNA, 321 bp, Artificial Sequence
gatatccagctgacccagagcccctcctttctgtccgcctccgtgggcgacagggtgaccatcacctgcagggccagctccaagacggggaacatccactggtatcaacagaagcctggcaaggcccccaagccctggatctacgccacctccaacctggccagcggcgtgcctagcaggttcagcggttctggctccggcaccgagttcaccctgaccatctcctccctgcagcccgaggacttcgccacctactactgccagcagtggtccagcaaccccctgacctttggccagggcaccaagctggagatcaagagg

SEQ ID NO: 44 - DNA, 30 bp, Artificial Sequence
agggccagctccaagacggggaacatccac

SEQ ID NO: 45 - protein, 107 aa, Artificial Sequence
DIQLTQSPSFLSASVGDRVTITCRASSKTGNIHWYQQKPGKAPKPWIYATSNLASGVPSRFSGSGSGTEFTLTISSLQPEDFATYYCQQWSSNPLTFGQGTKLEIKR

SEQ ID NO: 46 - protein, 10 aa, Artificial Sequence
RASSKTGNIH

SEQ ID NO: 47 - DNA, 642 bp, Artificial Sequence
gatatccagctgacccagagcccctcctttctgtccgcctccgtgggcgacagggtgaccatcacctgcagggccagctccggcgcgtccaacatccactggtatcaacagaagcctggcaaggcccccaagccctggatctacgccacctccaacctggccagcggcgtgcctagcaggttcagcggttctggctccggcaccgagttcaccctgaccatctcctccctgcagcccgaggacttcgccacctactactgccagcagtggtccagcaaccccctgacctttggccagggcaccaagctggagatcaagaggactgtggctgcaccatctgtcttcatcttcccgccatctgatgagcagttgaaatctggaactgcctctgttgtgtgcctgctgaataacttctatcccagagaggccaaagtacagtggaaggtggataacgccctccaatcgggtaactcccaggagagtgtcacagagcaggacagcaaggacagcacctacagcctcagcagcaccctgacgctgagcaaagcagactacgagaaacacaaagtctacgcctgcgaagtcacccatcagggcctgagctcgcccgtcacaaagagcttcaacaggggagagtgttaa

SEQ ID NO: 48 - protein, 213 aa, Artificial Sequence
DIQLTQSPSFLSASVGDRVTITCRASSGASNIHWYQQKPGKAPKPWIYATSNLASGVPSRFSGSGSGTEFTLTISSLQPEDFATYYCQQWSSNPLTFGQGTKLEIKRTVAAPSVFIFPPSDEQLKSGTASVVCLLNNFYPREAKVQWKVDNALQSGNSQESVTEQDSKDSTYSLSSTLTLSKADYEKHKVYACEVTHQGLSSPVTKSFNRGEC

SEQ ID NO: 49 - DNA, 321 bp, Artificial Sequence
gatatccagctgacccagagcccctcctttctgtccgcctccgtgggcgacagggtgaccatcacctgcagggccagctccggcgcgtccaacatccactggtatcaacagaagcctggcaaggcccccaagccctggatctacgccacctccaacctggccagcggcgtgcctagcaggttcagcggttctggctccggcaccgagttcaccctgaccatctcctccctgcagcccgaggacttcgccacctactactgccagcagtggtccagcaaccccctgacctttggccagggcaccaagctggagatcaagagg

SEQ ID NO: 50 - DNA, 30 bp, Artificial Sequence
agggccagctccggcgcgtccaacatccac

SEQ ID NO: 51 - protein, 107 aa, Artificial Sequence
DIQLTQSPSFLSASVGDRVTITCRASSGASNIHWYQQKPGKAPKPWIYATSNLASGVPSRFSGSGSGTEFTLTISSLQPEDFATYYCQQWSSNPLTFGQGTKLEIKR

SEQ ID NO: 52 - protein, 10 aa, Artificial Sequence
RASSGASNIH

SEQ ID NO: 53 - DNA, 97 bp, Artificial Sequence
ggggtaccgccgccaccatggagacagacacactcctgctatgggtactgctgctctgggttccaggttccactggtgaggtgcagctggtgcagag

SEQ ID NO: 54 - DNA, 34 bp, Artificial Sequence
ggctctagattatcactttccaggggacagtgac

SEQ ID NO: 55 - DNA, 97 bp, Artificial Sequence
ggggtaccgccgccaccatggagacagacacactcctgctatgggtactgctgctctgggttccaggttccactggtgatatccagctgacccagag

SEQ ID NO: 56 - DNA, 32 bp, Artificial Sequence
ggctctagattaacactctcccctgttgaagc